European Patent Application EP 4 303 309 A1, published January 10, 2024. Title: ERGOTHIONEINE PRODUCTION METHOD. Applicant: NAGASE & CO., LTD. The sequence listing filed with the application follows.

SEQUENCE LISTING (6 sequences)

SEQ ID NO: 1 - protein, 338 aa, Streptomyces coelicolor
MNRQPASPQERVHAVRIAVTGSIATDHLMTFPGRFSDQLVADQLHTVSLSFLVDQLDVRRGGVAANIAFGMGQLGTRPVLVGAAGSDFDEYRAWLDRHGVDTDSVRISETLHTARFVCTTDADHNQIGSFYTGAMSEARLIELKTVADRVGGLDLVSIGADDPEAMLRHTEECRARSIPFAADFSQQIARMNGDEIRILLDGATYLFSNEYEKGLIETKTGWSDAEILDRVGHRVTTLGARGVRIERAGGETIEVGVPDEERKADPTGVGDAFRAGFLSGLAWGVSLERAAQVGCMLATLVIETVGTQEYQLRRGHFMERFTKAYGDEAAGEVQAHLG

SEQ ID NO: 2 - DNA, 1017 bp, Artificial Sequence
  a nucleic aicf encoding an adenosine kinase from Streptomyces coelicolor optimized for E. coli
atgaatcggcaaccagcatctccgcaagaacgcgtgcatgcagtccgcattgcggtcaccggaagtatcgctaccgatcatctgatgacctttccaggacgcttctcggatcagttagtcgcggaccagcttcacaccgtgagcctgtcgtttctggtggatcagctcgatgttcgtcgcggaggcgtagccgccaacatcgcgttcggaatggggcaactgggtactcgtcctgtcctggttggtgccgctggcagtgacttcgacgaataccgcgcatggttagatcgccacggggtcgatacggactcagttcgcatttcggaaaccctgcatactgcgcgtttcgtatgcaccaccgatgctgatcacaaccagatcggctccttctatacaggtgccatgagcgaagcgcggctgattgagctgaaaacggttgcggatcgtgtaggcggtttggacctggtgagcattggcgcggatgaccccgaagcgatgttacgtcatacggaggagtgtcgcgcgcgctcaattccgtttgcggcggactttagccagcaaattgcccgcatgaatggcgacgaaattcgcattcttctggatggcgccacatacctcttcagcaacgagtacgagaagggcttgatcgaaacgaaaaccgggtggtccgacgccgaaatcttggatcgtgtgggtcatcgtgtgactacgctgggcgctcgtggggttcgtatcgaacgtgcaggcggtgaaaccatcgaagttggtgtaccggatgaagaacgcaaagcggatccgaccggtgtgggcgatgcgtttcgcgcaggctttctgtctggccttgcatggggtgtgagtctcgaacgcgctgcccaggttggttgcatgttagccaccctggtcattgagactgtgggtacacaggagtatcagctgcgtcgcggccactttatggaacggtttacgaaagcctatggcgatgaagcagcaggggaagtgcaagctcatctgggttaa

SEQ ID NO: 3 - DNA, 38 bp, Artificial Sequence
  primer
aacgaggcgcaaaaaatgaatcggcaaccagcatctcc

SEQ ID NO: 4 - DNA, 41 bp, Artificial Sequence
  primer
agctactagtctcgattaacccagatgagcttgcacttccc

SEQ ID NO: 5 - DNA, 47 bp, Artificial Sequence
  primer
cggccgctcatatgctcgaggtgactaattttccttgcggaggcttg

SEQ ID NO: 6 - DNA, 29 bp, Artificial Sequence
  primer
tttttgcgcctcgttatcatccaaaatac